European Patent Application EP 4 245 845 A1, published September 20, 2023. Title: Composition of decellularizated issue. Applicant: ADEKA CORPORATION. The sequence listing filed with the application follows.

SEQUENCE LISTING (3 sequences)

SEQ ID NO: 1 - protein, 339 aa, Bos taurus
MSTVHEILCKLSLEGDHSTPPSAYGSVKAYTNFDAERDALNIETAIKTKGVDEVTIVNILTNRSNEQRQDIAFAYQRRTKKELASALKSALSGHLETVILGLLKTPAQYDASELKASMKGLGTDEDSLIEIICSRTNQELQEINRVYKEMYKTDLEKDIVSDTSGDFRKLMVALAKGRRAEDGSVIDYELIDQDARDLYDAGVKRKGTDVPKWISIMTERSVCHLQKVFERYKSYSPYDMLESIKKEVKGDLENAFLNLVQCIQNKPLYFADRLYDSMKGKGTRDKVLIRIMVSRSEVDMLKIRSEFKKKYGKSLYYYIQQDTKGDYQKALLYLCGGDD

SEQ ID NO: 2 - protein, 375 aa, Bos taurus
MQWASILLLAGLCSLSWAQYEEDSHWWFQFLRNQQSTYDDPYDPYPYEPYEPYPTGEEGPAYAYGSPPQPEPRDCPQECDCPPNFPTAMYCDNRNLKYLPFVPSRMKYVYFQNNQISSIQEGVFDNATGLLWIALHGNQITSDKVGKKVFSKLRHLERLYLDHNNLTRIPSPLPRSLRELHLDHNQISRVPNNALEGLENLTALYLHHNEIQEVGSSMKGLRSLILLDLSYNHLRKVPDGLPSALEQLYLEHNNVFSVPDSYFRGSPKLLYVRLSHNSLTNNGLASNTFNSSSLLELDLSYNQLQKIPPVSTNLENLYLQGNRINEFSISSFCTVVDVMNFSKLQVQRLDGNEIKRSAMPADAPLCLRLASLIEI

SEQ ID NO: 3 - protein, 90 aa, Bos taurus
SNTFNSSSLLELDLSYNQLQKIPPVSTNLENLYLQGNRINEFSISSFCTVVDVMNFSKLQVQRLDGNEIKRSAMPADAPLCLRLASLIEI